European Patent Application EP 4 360 451 A1, published May 1, 2024. Title: MUTANTS FOR HAPLOID INDUCTION. Applicant: LIMAGRAIN EUROPE. Application EP. The sequence listing filed with the application follows.

SEQUENCE LISTING (27 sequences)

SEQ ID NO: 1 - protein, 380 aa, Zea mays
MLNLQLGIRHAVGKQGPITLDLKSSAFDPKEKVWTRFPPEGSKYTPPHSSCDFKWKDYCPQVFRTLRKLFKVDAADYMLSLCGDQALRELSSPGKSGSFFYLTSNDQYMIKTMKKSEVKIFLKMLRAYYNHVRSFESTLVTKFFGLHCVKLAGANQKKVRFVIMGNLFCSDYSIHRRFDLKGSSLGRTTDKPQTEIDEYTTLKDLDLNFIFRLQKHWYQEFQRQVDRDCEFLEQENIMDYSLLVGVHFRDTRDRLLTGGSFDSDCSRGSSPQLSRGDTDPNRLAKIKLGSNMPTRAERTIRKGDCEVQIMGEPTGEFYDVILYFGIIDILQDYDISKKLEHAYKSFQYDPTSISAVDPKQYSRRFRDFVFRAFQEDKFDL

SEQ ID NO: 2 - protein, 613 aa, Zea mays
MSSAAVSGSGGAAAAADGGVEGAPALSASASRTSSLRHRAMSASSKLLRSSLSRKSMGRRSSKVMSVSIEDVRDAEDMKQVDAFRQTLVLEELLPARHDDYHMMLRFLRARKFDIEKSKQMWSDMLQWRKEFGADTIIDEFVFEEMDQVLEHYPQGHHGVDKDGRPVYMEKLGQIDTTKLLQVTSMDRYVQYHVREFERAFAVKFPACSISAKKHVDQSTTILDVSGVGYKNFNKAARDLIGRLQKIDGDNYPETLCRMFIINAGQGFRLLWNTVKSFLDPKTTAKIHVLGNKYQSKLLEVIDASELPEFFGGTCNCEGGCMRSDKGPWKDPEILKMVQCGMGRCGMNSGDPRDADEKLITEDEIVPVPKKQDSMRRNAVDSPKVAREKIEHPQMSPLHEMKTASDPDPAAKDSFDGGGLFPGVDRGMDFNWSGEVSEEKLQIARDMYAQLPDAYKQGDAGDRQVVSGFMALVMGVVAMFRVGKIAPKRAMDAAMGIATMEAMAKKTRQMQMQQQLQLGGPDAVVVSAAQYQALVKRVDDLEAKVAALASGPPEVPPELEESIKAAAARVDALETELDATKKLLETSSAQQEEVLAYIEKKKKKRGMQNPFRW

SEQ ID NO: 3 - protein, 906 aa, Zea mays
MQRRSGDVRTPDAGFALLPTRFTIPDLLPLPTHGSPSIAMLRHCPHTCSQPSAFNPTGNVSSLDFLASFLPLSHSSVGDLISTGGMARILLHGSLHVTIFEAEELSNSSRPSSQAPGFLRKLVEGIEDTVGVGKGTSKIYATIGLGKTRVGRTRKLTDETASPRWYESFHVYCAHLASDVVFTIRAKNPIGASTVGVAYLPVRDIFEGHEVDRWLHLCDGGGDDKDRTPLESGGKVHVRLQYFDISKDHSWGKGVRSGKYPGVPYTFFSQRQGCRVTLYQDAHVPDGFVPRIPLDGGRCYEAHRCWEDIFDAISGAKHLIYITGWSVYTEITLLRDGARPPRPGSGVTLGELLKKKAGEGVRVLMLVWDDRTSVGALKKDGLMATHDEETMNYFEGTDVHCVLCPRNPDDSGSIVQDLQISTMFTHHQKIVVVDHDMPVQRSQRQRRILSFVGGLDLCDGRYDTPCHSLFRTLDGAHHDDFHQPNFATAAIAKGGPREPWHDIHCRLEGPVAWDVLYNFEQRWRKQGGKDLLIQLRDLADEIIAPSPVTFPNDPETWNVQLFRSIDGGAAFGFPDTPDDATRAGLVSGKDQIIDRSIQDAYIHAIRRARSFIYIENQYFLGSSYCWKPDGIKPEDIGALHVIPKELSMKVVSKIEAGERFAVYVVVPMWPEGIPESGSVQAILDWQRRTMEMMYTDIAQAIQAKGIDANPRDYLTFFCLGNREAKKPGEYVPTEEAEPDTGYIKAQQNRRFMIYVHTKMMMVDDEYIIVGSANINQRSMDGARDSEIAMGAYQPHHLAAASRPARGQVHGFRMSLWYEHLGAVDDAFTRPDSVECIRKVNAMADRYWDLYAGDGPERDLPGHLLTYPVAVGTDGSVNQLPGMEFFPDTQARVLGAKSDYLPPILTT

SEQ ID NO: 4 - protein, 596 aa, Zea mays
MGCGGSKEAVATGNSGSSRCNRFKRKSSVVDATQPSSRVLQPSLDNASAAAAAKASNGEVTKDKAATLKQKAVEEKKEEAVAVKNSKEAVSVKEGNAASSKASAIREEKPQVETKTDEAAAVTDAASEAAAAAVEKAGKEALAGKAAREKEGDEVVVVVKDKAVIAGQGLRIKHSSRTKQSSSTGGDVNAITVTAGKEEHIIRKDDVVKISTTEAAVDKGNNGGDEPDGTPYMAAIEENDDEAASSTEDVGDAVEEEDKKEVDDGSVTFPVSMVAEEDGSVTFKVRVNDAEAKDDDGSVKFATAAAGAAPTTSSNVVAVVAEEDGSVTFAVPVSPVIKDDDESVTSAAAPAAKVQDVVGAVVAEDDGSVTLAKPLAPVSVTKGGHSVSFVPARPATTKDDDDSVASAASPMTMDDEFVSLPVALEEEEEEEENEHWKDNDEAENEPAVSDDEEGTAEADGATEAEEDEEEAGQSEPSEDNDEVDDDADLPDPTAVEQLLTKAVEEIKAEEERSAADTVGENVSSKEPDEGKPIAPSRPRDEDGGEPDGKEPMDLEEEEARTTEEKTPDDHPGIPAEKKSGSDDKDSALPVSASSSS

SEQ ID NO: 5 - protein, 157 aa, Zea mays
MGDRHQHGPGSGVEDPATLLRRVQTRAPNSTQVVGFLTLLVSGAVLLLLTGVTLTGAVVALVFLGPIALLTSPIWVPVAVVISAIVAAALSACAFAAAALPVATWMYRYFTGRHPVGADRVDYARSRIADTASHVKDYAREYGGYLRTRAKDAAPGA

SEQ ID NO: 6 - protein, 146 aa, Zea mays
MPKNKGKGGKNRKRGKNEADDDKRELVFKEDGQEYAQVTRMLGNGRCEATCVDGTRRLCHIRGKMHKKVWIAAGDIVLVGLRDYQDDKADVILKYMNDEARLLKAYGELPETLRLNEGVDVDGPEEGEENGDYNYIQFEDEDIDKI

SEQ ID NO: 7 - protein, 633 aa, Zea mays
MTTVSSAAACLVLAVLLLPSAAQYVKYKDAKQPINERVQDLLGRMTLEEKIGQMSQIERANATAEVIEKYFVGSVLSGGGSVPAEKASASVWQKMVTRMQKAALKTRLGIPIIYGIDAVHGNNDVYNATIFPHNVGLGATRDPRLVKRVGEATAHETRATGIPYTFAPCVAVCRDPRWGRCYESFSEDTRLVQLMTSNMVAGLQGDVPAKHPKGVPFVGGAKKVAGCAKHFVGDGGTTRGINENNTVLSFHDLMRIHMPPYDNAVINGISSVMISYSSWNGVKMHENKFLITDTLKNKLNFRGFVITDWQAVDRITNPPHQHYYHSIKETIHAGIDMVMIPYDYPEFVADLAKQVKQGQIKLERIDDAVSRILRVKFAMGLFEDPLPDPRLTKELGAQEHRALAREAVRKSLVLLKNSKKGQAKPMLPLPKTAKKILVAGSHAHDLGSQCGGWTIKWQGERGNNLTGVGTTILEAIKKAVDKKTSVDYVERPDKDDLAKSAEGYEYAVVAVGEPPYAETAGDNKNLTIPSPGPEVIKDVCGLVRCVVLVVSGRPLVLQPYVDYMDALVAAWLPGTEAQGITDVLFGDYGFTGKLPRTWFKSVDQLPMNYGDKRYDPLFPFGFGLTTKAAASHD

SEQ ID NO: 8 - protein, 205 aa, Zea mays
MDRSNAGAVSVEVRGGGGGSPPGAGRKRRAVARGVQKTLSKTSMLANFLPTGTLLTFEMLLPAAAGDGTCSAVSAAMLRALLALCAASCFLFHFTDSFRAPDGKVYYGFVTPRGLSLFRTGLGVEVPREERYRLAFVDVVHAVMSVLVFAAVTLADYRVSGCLVAGHRKEMDEVMESFPLMVGAVCSGLFLLFPNTRYGIGCLAP

SEQ ID NO: 9 - protein, 542 aa, Zea mays
MLLHKGVAADEDLDEASRALLMKVLGDATQDAVRRQAKMLSGSLVSPALERELSMRSDCRTGHADPRLRPVASPSPRPSLLASERSRQLNLQHSTVSSRSGLHADGLHHAAEEPEEPTLALARLPFNRSSRTTLPAARHRPSQEQRHSNLSLHWFSVAGTSRHGTVTGSTPFANRRDSIYRSSGRGDQWALESSSRRRSVSRELSLGQSSRLHGRATIPRHVGADSSSSVPLFERLDSGLSVSMASLHGVERAGRGVATPERSSSSNTVATIRSRIRTSSTPFTERSLRRSAVQGRTPRSRGRQQGSDDVSSEDMYRSMYSGSRSSSCAASRSPTPPAPAPAPRAFANPYYYSPPVVTRGVAPPVYAPEQVSRSTRRRRRQEVLDKRVARLRMLKDKIGAVFHHRHDHHHHHHLGGGQEEGPSSRSRSVVRGAGHNSPWQFLTSMFHRAMEGKDKSTRIRTAVGVPAEKRRGGGGNMRALFDAVRRHLKGKRRAPAAGIKLRRKASLSRVRAKKMHWWQRLRRRRGMAGLTAGSRPRRRLGH

SEQ ID NO: 10 - protein, 492 aa, Arabidopsis thaliana
MEPNNVERNLQSLRRLYSLLVANARNEYIPEAYKLDDNTQFLLKRLLDFASHEHFVTQSNLLATQLRVFPKTVLHGAKPSNVADSSETTPPAMLSQINGSHITRVSKPLEAKGTLQRDLRVDQIRSNPSKDVLTEEVVDAIEQIDTQLSALSFVSSRVDSDERTRSVKSFVTPPTEECRQNSQASMPCLRSNYMTVSQKSVISGAEVTFPYNDQLVRVTSPPQPLPPRAVSGFKKPNQSNRASQKMPIMKPTLMDQETETFDDDSSETEADQTPSATGSESEDEEVSTSQEYSGETGSSSGSEWETQAENDTESKSESSYPPQNDDSVSEVSTSPPHTDRDTSREPGKQRRNVMGRFKRIKNKIGQIFHHHHHHHHHHHHHDKEKPSAWNKLQSKFHHKHQEKSKERKRPMSESKGLTTHKQQHQGGHFHALVEGLVRHRKHSKKQKHQLKSDAKKTEWWKLLKKRQGGGVKIPKRGRVKLGKKKHYLSKNV

SEQ ID NO: 11 - protein, 1093 aa, Zea mays
MANPAATSRRSALSSSPSPPPPLYLLLCLSLLLASTVQQPPTSQAQQVQAPEPAFMFGWLGNKREYTAGDTAAIRVMSLDHQAAAAVRATLSFTLSVNGKPGNSSYVTDVVANIGDDPSSWTVSFVPLRAGKFAALIGEPRFVPAEWPLTFTVAAAGVHPSASRASWTFADRRVVAGYRAFVSVFPRDTFGNGIARGPDMPGYFRVSGSYPNGSAVELLNFYYNGWIADGRIGLEFRTNVAGDFLVHVYGNDRELRDSPLMLTVDPGFLNIARSTCSWKHGINTLQLSSKLEMFIYQRDSFGNIVPEIHPFDAQVVDKATNLSIPIVDLAMEAVGDGVQLLSFNVVERGQFFLKVFDAKLNERVSNTVHSFDVFVGYCDGTKSFANGSGLANSIAGSTSSFSVFLKDFYNIPSPVETAKLQVKILGKYATSYVDPIISPVREPDGKLYANLAIIAGNSNMQTSKFNVSYTPQIAGEYEIWVLCGNIVLNGGNPYAMTVLPVAINTSLSRVVQFDPKVRLSIENEVVVRLVDSFMNPVESSKSKLKFRLTSASTTTPVTTTTSFVAKEFVNNSDGSYTGHYAAGGLGSYGICVLFEDKQLPPCPFEVTVHADEYFSDVKNDTVSVWEDESVSFDVLSNDRIAGSKAEIANSSSPLHGSVLQFGQTYRYTPFQGFFGNDSFSGFPGMKMVYSDTTENISVTVTAQSGSVSFDPVRIKLGQFSEDVLSISSRGGKDLVLQGTVEAVNGALDSLLYTGNEDFHGDDVVALNASSRNGVRRTQFPTFVEPINDPSVILAPSSILLSGNESWEGYRIFDKNRDTFEFSIVDPDIYNFPGKKSSFFLVLSLEVLEGTLTVTLPSSVIAAASMKTEAGSCWQPVQTYVTIANRFIVRGTAIRFRGSVRDCNRAMRQLRYYQGPTHGTTLSIAVNDQANHGCYPDCSERMTMPLSTAKTIRLVPLPVVAGALGHVSSRRAILFRWLAAAGIVVMLCQGCVLMCCLFKCMRALKSERRHKTYGQIRAPEQTAPFRQNMCASTSQREDVGYSPATATASQLGASRSSLRQRSPRSCNQEMELQPVSGAVNNRNEGSRPVSYKDK

SEQ ID NO: 12 - protein, 1065 aa, Zea mays
MGSGDDERSTSKHHHRDKDKDRDRSSSRHHRDKDRDRERSSRHHRDDGDRDRDRHHRDKDRDREERKEREREERKAREREERKAREREEREERDREKEKEKEKERARRREERDREERESSRRRGDADGEEDDDRDRKRRRRSSHHHHRDPEPEPEPASREEEEVDAEEAERRRQRKKEEDMEAEQQRLDDEMERRRRRVKEWQEKRREQQQQDGSVASGASAAVAAEADGAKAGKKWTLDGEESDEEEDKEDGKKAEGNGGAGDMDVGLPSGNGDANGGAEMEEDEIDPLDAFMNSMVLPEVAKLESAAVAMDTAPAAGADGKNGKSSKDVISNGDKKGSRKATGRIMQGDDSDSDYDDADDDGAGEDDEDDEEFIKRVKKTKAEKLAIVDHSKIDYQPFRKNFYIEVKDITKMTSEEVVDYRKHLELKVHGKDVPKPIKTWVQSGLTSKLLDTIKKLGFEKPMPIQTQALPIIMSGRDCIGIAKTGSGKTLAFVLPMLRHVKDQPPVVPGDGPIGLIMAPTRELVVQIHSDIKKFSKVLGINCVAIYGGSGVAQQISELKRGAEIVVCTPGRMIDILCTSSGKITNLRRVTFLVMDEADRMFDMGFEPQITRIVQNTRPDRQTVLFSATFPRQVEILARKVLTKPVEIQVGGRSVVNKDITQLVEVRPDTERFFRLLELLGEWYVKGKILVFVHSQDKCDSLLKDLFQHGYPCLSLHGGKDQTDRESTIADFKSNVCSLLIATSVAARGLDVKELELVVNYDVPNHYEDYVHRVGRTGRAGRKGFAVTFISDEDERYATDLVKALELSEQAVPQDLKALADRFMAKVKQGTEQAHGTGYGGSGFKFNEEEDEARKTAKKAQAREYGYEEDKSDSDSDDEGGVRKAGGDLAAQAIANAHAAAALVANKAANNANQQIPGSATAPLIPLLTASNQQNDEATARALQAAMNLQQNLARIQAHAVPEHYEAELEINDFPQNARWRITHKETLAPIQDWTGAAITTRGTYIPQGKIVGANERKLYLFIEGPTESSVKKAKAELKRVLEDCANQALNLPGSAQTGKYSVI

SEQ ID NO: 13 - protein, 895 aa, Zea mays
MASISLEDVRNETVDLETVPVQEVFQHLKCSKEGLSSAEGDNRLKIFGPNKLEEKSESKLLKFLGFMWNPLSWVMEAAAIMAIVLANGGGKPPDWQDFVGIVVLLFINSTISFIEENNAGNAAAALMAGLAPKTKVLRDGKWKEEEASILVPGDIISIKLGDIIPADARLLEGDPLKVDQAALTGESLPVNKHPGQGVFSGSTVKQGEIEAVVIATGVHTFFGKAAHLVDSTNNVGHFQLVLTAIGSHRLSQQGAITKRMTAIEEMAGMDVLCSDKTGTLTLNKLTVDKTLIEVCGKGVDKDMVLLYAARASRVENQDAIDTCIVGMLADPKEARAGIKEVHFLPFNPVEKRTAITYIDGNGDWHRVSKGAPEQIIELCRMSKDAEKKIHALIDGYADRGLRSLGVSYQLVPEKSKESAGEPWQFIGLLPLFDPPRHDSAETIRRALHLGVNVKMITGDQLAIGKETARRLGMGSNMYPSTTLLGDNKTGEMGGLNIDELIEKADGFAGVFPEHKYEIVKRLQDRKHICGMTGDGVNDAPALKKADIGIAVDDATDAARSASDIVLTEPGLSVIVSAVLTSRAIFQRMKNYTIYAVSITIRIVLGFLLVALVWKFDFAPFMVLIIAILNDGTIMTISKDRVKPSPTPDSWKLKEIFATGIVLGTYMALATALFFYLAHDTDFFTNAFGVRSIKENDKELMAALYLQVSIISQALIFVTRSRSWSFVERPGALLVIAFLAAQLVATCIAVYANWEFCKMQGIGWGWGGAIWAFSVVTYFPLDVLKFAIRYALSGKAWNNINNKTAFTNRTDYGKGEREAQWATAQRTLHGLNQATATSDLFGDNQGYRELSELAEQAAKRAEVARLRELHTLKGHVESVVKLKGLDIDTIQQSYTV

SEQ ID NO: 14 - protein, 248 aa, Zea mays
MGKGGGCVPSKKRQPPAAAPSSSSAAAAVPREAPEEEAAAAVGRKLRLYIVFYSMYGHVESLARRAAAGAGAVDGLEAVLRRVPETLPPEVLEKMQAPVKDPAVPVIASAAELQEADGVLFGFPTRYGAMAAQMKAFFDSTGSLWEAQKLAGKPAGFFVSTGTQGGGQETTAWTAITQLAHHGMLFVPIGYTFGSGMFDMDGIRGGSPYGAGVFAGDGSRQPSETELALAEHQGKYMASIVKKLALHA

SEQ ID NO: 15 - protein, 1103 aa, Zea mays
MPALKVLRFPLASPPDGPPSKTPPALSVSRAPPPQYHFVRKNKGESSRKSSPPPASPPLLPVIAPPPERPSRGRVVGFGAGPGPGPDPPMASTEQEAAVEAAAVVEEVTRQQGKGCGVAGGGDTVGSWRNIDIAWRKADEAAIRRYEAANWLRRIVGVVCAKDLAEEPSEEEFRIGLRNGIILCNALNKIQPGAVPKVVEVPSDSTAPVDGTALCAYQYFENVRNFLTGMQDLGLTTFEASDLEKGGQGVRVVDCVLAMKSFCDAKHVGKRSPFKYGGIVKPLSGKYVIRKNNEPYMKVMMRSHSAELLRDGISLEQIGLDFSLEPTETTATPDSIRMLVQTVLADKKPEEIPSVVESLLSKVINEYDCRIASQSEVVKDTMEQVKDTMEQVKDTMDTNDCNSVLRMDSPFDTNDTKSLSRVDSPQVESTTPSDLDKATENIKMDEDEQNASSLTEDVSTLVPLPVPVPLSNDIVINIPKIVRNFDQEEKQIQDLKSNMSTVKSFMEQLKLLYSEDLKKLGDHLRIISHAASGYRKVVEENRKLYNQIQDLRGNIRVYCRVRPFHPGKEFPSSSVAGIEDRTITVMVPSKHGKDGKKSFTFNSVFGPLATQADVFTDMQPLVRSVLDGFNVCIFAYGQTGSGKTFTMSGPKILTEEGLGVNYRALNDLFGIQEQRKDTICYEIAVQMMEIYNEQVRDLLQTGGNKKYPFTLSLILILLLDILTFFFLHMLNIYLIYVGLLNAKKHWKFEIILKTELQFQMQMWCHCLTVHVQGRDLTSGTVLRGCMHLVDLAGSERVDKSEVVGIGLKEAQHINKSLAALGDVIAALAQKSTHVPYRNSKLTQLLQDSLGGQAKTLMFIHIAPEPDAISESISTLKFAERVSTIELGAAKSSKEGGGGGGGEARELKEQIACLRAALARKDGDHESIRSTQSSPDIYRMGTGNASPASRHPIEDGIIENDSALGDLAEHSQFGSSNSLPELGPDATQDLAFYQRSNSEQQWSWSGSVATEDSDDFEVATNCSLELDCVRPSSAPKASGLSNGGGTAVKKIQVKGSKGSDVRGVNPGKRSSPLQKKPSGPSPTLIKKGGGEGRKTPNGKTGTKK

SEQ ID NO: 16 - DNA, 2062 bp, Zea mays
  source 1..2062: mol_type = other DNA
  misc_feature 1..2062: gene = ZmKpla_cri-1_Zm00001d002427_T001_V4
atgctgcttcacaagggtgttgctgcagatgaagatgtaaggatttttttcatggcttcactgttgtcttgtgagaagcgagagagaactcgaagacattaagacaggttttgtttttagtgaaaactaaattcaggcatggtagaccctaaaccgaagcaatacttctgatttccatatctcactgactaactgcaagcatggagcaaaactgaagcgatgcgaaccaatttcgatgtttgttttgcgagaccaaaagttcaaagtctaaagtttttttttctgtgggagagaaatacgtttgcagtgtaatgcaaacagtcgctttgttcttgttcttgcttttgtgcagttagatgaggcatccagggctctcctgatgaaggtactaggagatgccacccaggacgctgtgcggaggcaggcaaaggtaacctgttttttttcttttcttgttgtgccattaattgtagacggccacaccttcacagtactatcttctggtgaaatgccaacgccaaccaaaattaagatttgtctttctgcagatgttatcaggttctctagtgtccccagcgctagagagagagctctccatgcgatcagactgccggacgggcatgccgatccgcgcctgaggccagtggcgtcacccagtcccagacccagcctcctggccagtgagcgatcgcgccagcttaacctgcaacactctacggtgtcaagccgatccggcctccacgccgacggccttcaccatgcagcggaagagcctgaagagcctacccttgcccttgctcgcctccccttcaatcgctcgtcgagaaccacgttgccggcagcacggcatcgtccaagccaagagcaacggcactccaacctcagcctccactggttctccgtggctggaacgtcgagacatggcacggtgaccggaagtactccgtttgccaaccgccgggacagtatctatcgcagctctggccgtggtgaccagtgggcgctggaaagcagcagcaggcggcgttccgtgtcgcgtgagctgtctctggggcaatcgtcaaggctgcatggccgcgccaccatcccgcggcacgtgggagcggatagctcctcctcggtgcctctcttcgagaggctggactctgggctgtccgtgagcatggcgtcgcttcatggcgtggagcgtgccggacgcggcgtggctacgccggaacgctcttcctcgagcaacacggtggcgaccattcgaagccgcatcagaacaagcagcactcctttcacggagcgctccctgcgccgatcagcagtacaagggaggactccacgttcacgcgggaggcaacaaggcagcgacgacgtttccagcgaggacatgtaccgcagcatgtacagcggtagcagaagctcatcgtgcgccgcctccagaagcccgacgccgccggcgccggcgccggcgccgcgtgcttttgctaacccctactactactcgccgccggtggtgacacggggcgttgctccgccggtgtacgcacctgagcaggtgtcgcgctcaacgaggaggcgtcgtcgacaggaagtcctggacaagcgggtggcgcggctgcggatgctcaaggacaaaatcggcgcggtgttccatcaccgccacgaccatcaccaccaccaccacctcgggggcggccaggaggagggcccctcgtccaggtccaggagcgtcgtccgcggcgcgggccacaactcgccgtggcagttccttacgagcatgttccaccgcgcgatggaagggaaagataagagcacgaggatccgaacggcggtaggcgtgccggcggagaagaggcgcggcggtggcgggaacatgcgcgctctctttgacgcggtccggcggcacctgaagggaaagcggagggcaccggcggcaggcataaagctgaggaggaaggccagcctgagccgggtgcgggccaagaagatgcattggtggcagcggctgaggcggcggcgcggcatggcagggctgacggcgggcagtagaccacggcgccgtttaggacattga

SEQ ID NO: 17 - DNA, 2379 bp, Zea mays
  source 1..2379: mol_type = other DNA
  misc_feature 1..2379: gene = ZmKplb_cri-1_Zm00001d026242_T001_V4
atggatcgtgcgacgtcgtcgagttcgtcatttcttaacaacagtgagtggtcgttgaaccgatctttgttcttggctgtctttccatccctcccggcatttctccttgcggggaaagatacatgtctctgtggcaatgagttttgttactcatttcttgttctaatttcgaaatgggtagagttgcctgaagaaacagcgatggagcaaattttgactgatctgcaggcgctcacgaggctatacggcctgcttcacagtccagcagacgaaaatgtaagggaattttttttttggcttctctgctatgtcttgtgacgagtgagaaaagtatattttgttgtttagtagaaactaaatttaggcatggtaaaccgaagcaatagttctactttcaatatgtaactgcaaggctgaggtgtaaaactgaagctgatctgagcgagccagtttcaacgtttattttgcgagatcgaagtcctcagtttttctgcgatagagaaatatgtttgcgcatttcatgtaaacagccgcaagtttgatctgttcttagtttttatgcagttagatgaggcatccagggctcttctgatgaagatactagaagatgctacccaggaggctgtccggaggcaggcgaaggtatcgatgcattttaactgtagacggccacaccttcacagcacttatttttctggtcaaaatgccaatgatcttcaaatttaaaatttccctttctgcagatgctaatgccatcaggttctctaatgtcccctgtgctagagagagagctctccacacaatcacactgccggacacgccatgccgatccaatcactgaggccactggcctcgccccgccccagcctcctggccagtgagcgatcgcgccggctagacccgcaacattctacagtgtcacgccgatccggcctctacgccgacggccagcgccatgcagcggaagagcctcctccccttgctcgcctcgcctccaaccgctcgtcgagaaccgcattgacggcgcggcaccgtccaagccaagagcagcggtgccccagcctcagcctgcaccgtttccccgtagctggaacgtcgagacatggcacggtgatcggaagtactcggcttgcccgtcgccgggacagcatccgtcacagctccggtcgtggtgaccagtggtcgctggaacgcagcaatagcaatagcagcagcagccgccgttccgtgtcacggcgagagctgtcgtctctgcggccgtcgtcaaggctgcgtggccgcgccaccccgcggcacgtgggaacggaaaactcctcctcggtgtctcccttcgagaggctggactctgggttgtccctgagcttgacgtcgcgtcatggcgtggagcatgccggacgcggcgtggctacgccggaacgctcttcctcgagcaagacggtggcgaccattcaaagccgcatccgaccaagcagtactcctctcagggagcgctccctacaccgacctgcagtagaagcgaagactctgcgcgggaggcaacaagacagccacgttttaagcgaggaggacacgtacagcagcatgttcagcggcagcggaagctcatcggacgccgccagcctgtccgcctccacgagcccgacggcgtcgccggcgccggcgccggcgccgcgtgcttctgctactccctactactactacccgtcggtggcgacacgtggcattgcgccaccaccgttgtacgcacctgaggtgtcgcgctcaatgaggaggcgacgtctccaggaacgtcggcaggaaatcctggagaggcgggtggcgcggctgcggatgctcaagaacaaaatcgccacggtgttccatgacttccatcaccgccacgaccaccaccaccacctcctcctcgggggcggccaggaggcgggtccctcgtccaggactgtcgtccgcggcgcaggccaccaccaccacctcgggggcggccaggaggcgggcccctcgtctagggccgtcgtccgcggcgcaggccaccacctcaactcgccgtggcagtaccttacgagaatgttccaccgcgcgaaagggaagatagacaagaatactaggagccggacggcggtaggcgtgccggaaaagaggcacggcgctggcggtggcggtggcgggaacatgcacgcgctattcgacgcgctgcggcggcacctgaagagcaagcggagggcaccggcaggcataaaactggggaggaagggcaactgggtgcggggcaagaagatgcattggtggcagcggctgaggcgacggcgcggcatgccagggttgacggcaggcagtggaccacggcggcgtttacgacatggaaaggcagcgtggctgtag

SEQ ID NO: 18 - DNA, 2376 bp, Zea mays
  source 1..2376: mol_type = other DNA
  misc_feature 1..2376: gene = ZmKplb_cri-2_Zm00001d026242_T001_V4
atggatcgtgcgacgtcgtcgagttcgtcatttcttaacaacagtgagtggtcgttgaaccgatctttgttcttggctgtctttccatccctcccggcatttctccttgcggggaaagatacatgtctctgtggcaatgagttttgttactcatttcttgttctaatttcgaaatgggtagagttgcctgaagaaacagcgatggagcaaattttgactgatctgcaggcgctcacgaggctatacggcctgcttcacagtccagcagacgaaaatgtaagggaattttttttttggcttctctgctatgtcttgtgacgagtgagaaaagtatattttgttgtttagtagaaactaaatttaggcatggtaaaccgaagcaatagttctactttcaatatgtaactgcaaggctgaggtgtaaaactgaagctgatctgagcgagccagtttcaacgtttattttgcgagatcgaagtcctcagtttttctgcgatagagaaatatgtttgcgcatttcatgtaaacagccgcaagtttgatctgttcttagtttttatgcagttagatgaggcatccagggctcttctgatgaagatactagaagatgctacccaggaggctgtccggaggcaggcgaaggtatcgatgcattttaactgtagacggccacaccttcacagcacttatttttctggtcaaaatgccaatgatcttcaaatttaaaatttccctttctgcagatgctaatgccatcaggttctctaatgtcccctgtgctagagagagagctctccacacaatcacactgccggacacgccatgccgatccaactgaggccactggcctcgccccgccccagcctcctggccagtgagcgatcgcgccggctagacccgcaacattctacagtgtcacgccgatccggcctctacgccgacggccagcgccatgcagcggaagagcctcctccccttgctcgcctcgcctccaaccgctcgtcgagaaccgcattgacggcgcggcaccgtccaagccaagagcagcggtgccccagcctcagcctgcaccgtttccccgtagctggaacgtcgagacatggcacggtgatcggaagtactcggcttgcccgtcgccgggacagcatccgtcacagctccggtcgtggtgaccagtggtcgctggaacgcagcaatagcaatagcagcagcagccgccgttccgtgtcacggcgagagctgtcgtctctgcggccgtcgtcaaggctgcgtggccgcgccaccccgcggcacgtgggaacggaaaactcctcctcggtgtctcccttcgagaggctggactctgggttgtccctgagcttgacgtcgcgtcatggcgtggagcatgccggacgcggcgtggctacgccggaacgctcttcctcgagcaagacggtggcgaccattcaaagccgcatccgaccaagcagtactcctctcagggagcgctccctacaccgacctgcagtagaagcgaagactctgcgcgggaggcaacaagacagccacgttttaagcgaggaggacacgtacagcagcatgttcagcggcagcggaagctcatcggacgccgccagcctgtccgcctccacgagcccgacggcgtcgccggcgccggcgccggcgccgcgtgcttctgctactccctactactactacccgtcggtggcgacacgtggcattgcgccaccaccgttgtacgcacctgaggtgtcgcgctcaatgaggaggcgacgtctccaggaacgtcggcaggaaatcctggagaggcgggtggcgcggctgcggatgctcaagaacaaaatcgccacggtgttccatgacttccatcaccgccacgaccaccaccaccacctcctcctcgggggcggccaggaggcgggtccctcgtccaggactgtcgtccgcggcgcaggccaccaccaccacctcgggggcggccaggaggcgggcccctcgtctagggccgtcgtccgcggcgcaggccaccacctcaactcgccgtggcagtaccttacgagaatgttccaccgcgcgaaagggaagatagacaagaatactaggagccggacggcggtaggcgtgccggaaaagaggcacggcgctggcggtggcggtggcgggaacatgcacgcgctattcgacgcgctgcggcggcacctgaagagcaagcggagggcaccggcaggcataaaactggggaggaagggcaactgggtgcggggcaagaagatgcattggtggcagcggctgaggcgacggcgcggcatgccagggttgacggcaggcagtggaccacggcggcgtttacgacatggaaaggcagcgtggctgtag

SEQ ID NO: 19 - DNA, 2377 bp, Zea mays
  source 1..2377: mol_type = other DNA
  misc_feature 1..2377: gene = ZmKplb_cri-3_Zm00001d026242_T001_V4
atggatcgtgcgacgtcgtcgagttcgtcatttcttaacaacagtgagtggtcgttgaaccgatctttgttcttggctgtctttccatccctcccggcatttctccttgcggggaaagatacatgtctctgtggcaatgagttttgttactcatttcttgttctaatttcgaaatgggtagagttgcctgaagaaacagcgatggagcaaattttgactgatctgcaggcgctcacgaggctatacggcctgcttcacagtccagcagacgaaaatgtaagggaattttttttttggcttctctgctatgtcttgtgacgagtgagaaaagtatattttgttgtttagtagaaactaaatttaggcatggtaaaccgaagcaatagttctactttcaatatgtaactgcaaggctgaggtgtaaaactgaagctgatctgagcgagccagtttcaacgtttattttgcgagatcgaagtcctcagtttttctgcgatagagaaatatgtttgcgcatttcatgtaaacagccgcaagtttgatctgttcttagtttttatgcagttagatgaggcatccagggctcttctgatgaagatactagaagatgctacccaggaggctgtccggaggcaggcgaaggtatcgatgcattttaactgtagacggccacaccttcacagcacttatttttctggtcaaaatgccaatgatcttcaaatttaaaatttccctttctgcagatgctaatgccatcggttctctaatgtcccctgtgctagagagagagctctccacacaatcacactgccggacacgccatgccgatccaatcctgaggccactggcctcgccccgccccagcctcctggccagtgagcgatcgcgccggctagacccgcaacattctacagtgtcacgccgatccggcctctacgccgacggccagcgccatgcagcggaagagcctcctccccttgctcgcctcgcctccaaccgctcgtcgagaaccgcattgacggcgcggcaccgtccaagccaagagcagcggtgccccagcctcagcctgcaccgtttccccgtagctggaacgtcgagacatggcacggtgatcggaagtactcggcttgcccgtcgccgggacagcatccgtcacagctccggtcgtggtgaccagtggtcgctggaacgcagcaatagcaatagcagcagcagccgccgttccgtgtcacggcgagagctgtcgtctctgcggccgtcgtcaaggctgcgtggccgcgccaccccgcggcacgtgggaacggaaaactcctcctcggtgtctcccttcgagaggctggactctgggttgtccctgagcttgacgtcgcgtcatggcgtggagcatgccggacgcggcgtggctacgccggaacgctcttcctcgagcaagacggtggcgaccattcaaagccgcatccgaccaagcagtactcctctcagggagcgctccctacaccgacctgcagtagaagcgaagactctgcgcgggaggcaacaagacagccacgttttaagcgaggaggacacgtacagcagcatgttcagcggcagcggaagctcatcggacgccgccagcctgtccgcctccacgagcccgacggcgtcgccggcgccggcgccggcgccgcgtgcttctgctactccctactactactacccgtcggtggcgacacgtggcattgcgccaccaccgttgtacgcacctgaggtgtcgcgctcaatgaggaggcgacgtctccaggaacgtcggcaggaaatcctggagaggcgggtggcgcggctgcggatgctcaagaacaaaatcgccacggtgttccatgacttccatcaccgccacgaccaccaccaccacctcctcctcgggggcggccaggaggcgggtccctcgtccaggactgtcgtccgcggcgcaggccaccaccaccacctcgggggcggccaggaggcgggcccctcgtctagggccgtcgtccgcggcgcaggccaccacctcaactcgccgtggcagtaccttacgagaatgttccaccgcgcgaaagggaagatagacaagaatactaggagccggacggcggtaggcgtgccggaaaagaggcacggcgctggcggtggcggtggcgggaacatgcacgcgctattcgacgcgctgcggcggcacctgaagagcaagcggagggcaccggcaggcataaaactggggaggaagggcaactgggtgcggggcaagaagatgcattggtggcagcggctgaggcgacggcgcggcatgccagggttgacggcaggcagtggaccacggcggcgtttacgacatggaaaggcagcgtggctgtag

SEQ ID NO: 20 - DNA, 2377 bp, Zea mays
  source 1..2377: mol_type = other DNA
  misc_feature 1..2377: gene = ZmKplb_cri-4_Zm00001d026242_T001_V4
atggatcgtgcgacgtcgtcgagttcgtcatttcttaacaacagtgagtggtcgttgaaccgatctttgttcttggctgtctttccatccctcccggcatttctccttgcggggaaagatacatgtctctgtggcaatgagttttgttactcatttcttgttctaatttcgaaatgggtagagttgcctgaagaaacagcgatggagcaaattttgactgatctgcaggcgctcacgaggctatacggcctgcttcacagtccagcagacgaaaatgtaagggaattttttttttggcttctctgctatgtcttgtgacgagtgagaaaagtatattttgttgtttagtagaaactaaatttaggcatggtaaaccgaagcaatagttctactttcaatatgtaactgcaaggctgaggtgtaaaactgaagctgatctgagcgagccagtttcaacgtttattttgcgagatcgaagtcctcagtttttctgcgatagagaaatatgtttgcgcatttcatgtaaacagccgcaagtttgatctgttcttagtttttatgcagttagatgaggcatccagggctcttctgatgaagatactagaagatgctacccaggaggctgtccggaggcaggcgaaggtatcgatgcattttaactgtagacggccacaccttcacagcacttatttttctggtcaaaatgccaatgatcttcaaatttaaaatttccctttctgcagatgctaatgccatcaggttctctaatgtcccctgtgctagagagagagctctccacacaatcacactgccggacacgccatgccgatccaatctgaggccactggcctcgccccgccccagcctcctggccagtgagcgatcgcgccggctagacccgcaacattctacagtgtcacgccgatccggcctctacgccgacggccagcgccatgcagcggaagagcctcctccccttgctcgcctcgcctccaaccgctcgtcgagaaccgcattgacggcgcggcaccgtccaagccaagagcagcggtgccccagcctcagcctgcaccgtttccccgtagctggaacgtcgagacatggcacggtgatcggaagtactcggcttgcccgtcgccgggacagcatccgtcacagctccggtcgtggtgaccagtggtcgctggaacgcagcaatagcaatagcagcagcagccgccgttccgtgtcacggcgagagctgtcgtctctgcggccgtcgtcaaggctgcgtggccgcgccaccccgcggcacgtgggaacggaaaactcctcctcggtgtctcccttcgagaggctggactctgggttgtccctgagcttgacgtcgcgtcatggcgtggagcatgccggacgcggcgtggctacgccggaacgctcttcctcgagcaagacggtggcgaccattcaaagccgcatccgaccaagcagtactcctctcagggagcgctccctacaccgacctgcagtagaagcgaagactctgcgcgggaggcaacaagacagccacgttttaagcgaggaggacacgtacagcagcatgttcagcggcagcggaagctcatcggacgccgccagcctgtccgcctccacgagcccgacggcgtcgccggcgccggcgccggcgccgcgtgcttctgctactccctactactactacccgtcggtggcgacacgtggcattgcgccaccaccgttgtacgcacctgaggtgtcgcgctcaatgaggaggcgacgtctccaggaacgtcggcaggaaatcctggagaggcgggtggcgcggctgcggatgctcaagaacaaaatcgccacggtgttccatgacttccatcaccgccacgaccaccaccaccacctcctcctcgggggcggccaggaggcgggtccctcgtccaggactgtcgtccgcggcgcaggccaccaccaccacctcgggggcggccaggaggcgggcccctcgtctagggccgtcgtccgcggcgcaggccaccacctcaactcgccgtggcagtaccttacgagaatgttccaccgcgcgaaagggaagatagacaagaatactaggagccggacggcggtaggcgtgccggaaaagaggcacggcgctggcggtggcggtggcgggaacatgcacgcgctattcgacgcgctgcggcggcacctgaagagcaagcggagggcaccggcaggcataaaactggggaggaagggcaactgggtgcggggcaagaagatgcattggtggcagcggctgaggcgacggcgcggcatgccagggttgacggcaggcagtggaccacggcggcgtttacgacatggaaaggcagcgtggctgtag

SEQ ID NO: 21 - DNA, 2541 bp, Zea mays
  source 1..2541: mol_type = other DNA
  misc_feature 1..2541: gene = Zm00001d015175_B73_C5175_cri-2_T001_V4
atgtcgtccgcagccgtgtcgggcagcggcggcgccgccgccgcggcggacggcggcgtggagggcgcgccggcgctgtcggcgtcggcgtcgcgcacgtcgtcgctgcggcaccgcgcgatgagcgcgtcgtcgaagctgctgcggagctcgctgagccgcaagtcgatggggcggcgcagcagcaaggtgatgtcggtgtcgatcgaggacgtgcgcgacgcggaggatatgaagcaggtggacgcgttccggcagacgctggtgctggaggagctgctgccggcccgccacgacgactaccacatgatgctccggttcctgcgcgcgcgcaagttcgacatcgagaagtcgaagcagatgtggtcggacatgctgcagtggcgcaaggagttcggcgccgacaccatcatcgacgagttcgtgttcgaggagatggaccaggtgctggagcactacccgcagggccaccacggcgtggacaaggacggccggcccgtgtacatggagaagctggggcagatcgacaccaccaagctgctgcaggtcaccagcatggaccgctacgtgcagtaccagtgagggagttcgagcgcgccttcgccgtcaagttccccgcctgctccatctccgccaagaagcacgtcgaccagagcaccaccatccttgacgtctccggcgtggtccgtgtcccgagtctccaccaccatccgtctcttgctgctcgctgctgcttgatgctttcttctcatccatggcgtgcgccattgttgcccaggggtacaagaacttcaacaaggccgcgagggacctcatcggacgcctccagaagatcgacggagacaactaccctgaggtaccacactgcatgtcctgttcgatcgtccagtgaacttgttcgtccaagcaactgcaacaagtgcagccttctgctacatgctcgccctgtgcagacgctgtgccggatgttcatcatcaacgcggggcaagggttcaggcttctctggaacaccgtcaagtcgttcctggaccccaagaccacggccaagatccatgtaaccaaaccgatttctcctccccctcccatcacaggcattggttggttccactcacttgatcatctgctctgctctgctctgatggcggtgcaggtccttggcaacaagtaccagagcaagctcctggaagtgatcgatgccaggtttatttgctgaacaaactggactgaactcactgctcaggtttctttcttgacctctttgtgatgacgtgtgtgcagcgagctgcccgagttcttcggcggcacttgcaactgcgagggcggctgcatgcgctccgacaaagggccatggaaggaccctgagatcctcaaggttccgtctacctgtctagattactttgcgctccactccgacgaagggccagccatgtgaagctggtagacgatcgatgctgtttttcatccggttctttctcagatggtccaatgcggcatggggagatgcgggatgaacagcggggaccctcgcgacgccgacgagaagctcatcaccgaggacgaaatagtgcccgttcccaaggtacggtgtgtgtgtgtttgtcatcaagcctgaacagcaagcaacacatggagcatgcaacgcgcagaacagaacgctgtgtcactgacagtgacaccggtttccgatccacactgcagaagcaagactccatgcgccgcaacgccgtggattcccccaaggtggcgcgcgagaagatcgagcacccgcagatgtccccgctccacgagatgaagaccgccagcgacccggaccctgccgccaaggacagcttcgacggcggcgggctgttccccggcgtggacaggggcatggacttcaactggagcggcgaggtgagcgaggagaagctgcagatcgcgcgggacatgtacgcgcagctgccggacgcgtacaagcagggggacgcgggagaccggcaggtggtgtcggggttcatggcgctggtgatgggcgtggtggccatgttccgggtgggcaagatcgcgccgaagcgggccatggacgcggccatgggcatcgccaccatggaggccatggccaagaagacgcggcagatgcagatgcagcagcagctgcagctgggcgggcccgacgccgtcgtggtgtcggcggcgcagtaccaggcgctggtcaagcgcgtggacgacctggaggccaaggtggcggcgctggcgtcgggcccgcccgaggtgccgcccgagctggaggagtcgatcaaggccgccgccgcccgcgtcgacgcgctcgagacggagctcgacgccaccaagaagctactcgagacgtcgtccgcccagcaggaggaggtcctggcgtacatcgagaagaagaagaagaagcgagggatggtaagtcagtccagtccagtccagtccagtgtgtttctgatcttggcgttggctgccactccgcggttgatttgtgtgagctgatttcattaaagttttgcctccaacagcagaacccgttccgatggtga

SEQ ID NO: 22 - DNA, 2424 bp, Zea mays
  source 1..2424: mol_type = other DNA
  misc_feature 1..2424: gene = Zm00001d015175_B73_C5175_cri-3_T001_V4
atgtcgtccgcagccgtgtcgggcagcggcggcgccgccgccgcggcggacggcggcgtggagggcgcgccggcgctgtcggcgtcggcgtcgcgcacgtcgtcgctgcggcaccgcgcgatgagcgcgtcgtcgaagctgctgcggagctcgctgagccgcaagtcgatggggcggcgcagcagcaaggtgatgtcggtgtcgatcgaggacgtgcgcgacgcggaggatatgaagcaggtggacgcgttccggcagacgctggtgctggaggagctgctgccggcccgccacgacgactaccacatgatgctccggttcctgcgcgcgcgcaagttcgacatcgagaagtcgaagcagatgtggtcggacatgctgcagtggcgcaaggagttcggcgccgacaccatcatcgacgagttcgtgttcgaggagatggaccaggtgctggagcactacccgtgagggagttcgagcgcgccttcgccgtcaagttccccgcctgctccatctccgccaagaagcacgtcgaccagagcaccaccatccttgacgtctccggcgtggtccgtgtcccgagtctccaccaccatccgtctcttgctgctcgctgctgcttgatgctttcttctcatccatggcgtgcgccattgttgcccaggggtacaagaacttcaacaaggccgcgagggacctcatcggacgcctccagaagatcgacggagacaactaccctgaggtaccacactgcatgtcctgttcgatcgtccagtgaacttgttcgtccaagcaactgcaacaagtgcagccttctgctacatgctcgccctgtgcagacgctgtgccggatgttcatcatcaacgcggggcaagggttcaggcttctctggaacaccgtcaagtcgttcctggaccccaagaccacggccaagatccatgtaaccaaaccgatttctcctccccctcccatcacaggcattggttggttccactcacttgatcatctgctctgctctgctctgatggcggtgcaggtccttggcaacaagtaccagagcaagctcctggaagtgatcgatgccaggtttatttgctgaacaaactggactgaactcactgctcaggtttctttcttgacctctttgtgatgacgtgtgtgcagcgagctgcccgagttcttcggcggcacttgcaactgcgagggcggctgcatgcgctccgacaaagggccatggaaggaccctgagatcctcaaggttccgtctacctgtctagattactttgcgctccactccgacgaagggccagccatgtgaagctggtagacgatcgatgctgtttttcatccggttctttctcagatggtccaatgcggcatggggagatgcgggatgaacagcggggaccctcgcgacgccgacgagaagctcatcaccgaggacgaaatagtgcccgttcccaaggtacggtgtgtgtgtgtttgtcatcaagcctgaacagcaagcaacacatggagcatgcaacgcgcagaacagaacgctgtgtcactgacagtgacaccggtttccgatccacactgcagaagcaagactccatgcgccgcaacgccgtggattcccccaaggtggcgcgcgagaagatcgagcacccgcagatgtccccgctccacgagatgaagaccgccagcgacccggaccctgccgccaaggacagcttcgacggcggcgggctgttccccggcgtggacaggggcatggacttcaactggagcggcgaggtgagcgaggagaagctgcagatcgcgcgggacatgtacgcgcagctgccggacgcgtacaagcagggggacgcgggagaccggcaggtggtgtcggggttcatggcgctggtgatgggcgtggtggccatgttccgggtgggcaagatcgcgccgaagcgggccatggacgcggccatgggcatcgccaccatggaggccatggccaagaagacgcggcagatgcagatgcagcagcagctgcagctgggcgggcccgacgccgtcgtggtgtcggcggcgcagtaccaggcgctggtcaagcgcgtggacgacctggaggccaaggtggcggcgctggcgtcgggcccgcccgaggtgccgcccgagctggaggagtcgatcaaggccgccgccgcccgcgtcgacgcgctcgagacggagctcgacgccaccaagaagctactcgagacgtcgtccgcccagcaggaggaggtcctggcgtacatcgagaagaagaagaagaagcgagggatggtaagtcagtccagtccagtccagtccagtgtgtttctgatcttggcgttggctgccactccgcggttgatttgtgtgagctgatttcattaaagttttgcctccaacagcagaacccgttccgatggtga

SEQ ID NO: 23 - DNA, 4311 bp, Zea mays
  source 1..4311: mol_type = other DNA
  misc_feature 1..4311: gene = Zm00001d016601_B73_P6601_cri-8_T004_V4
atggcagaagtcctatcaggatctcatgaacaccgtctaagctctggtgagtatgcatataattaaatgacatgaccattctcttgctgactgagatggataatatattgcaacagtactttctttctttctttgccctcataaaaaaacttgtgatattcctgtaatgtctgatttttttattgaaacgttgcacttatggcaacacatttttgttttccccaataatcatggacaatttagcataatccatgcaagtcaaattcagtccccgaaattaaacttcacagaattgacttatctagaaatgatatctgcagccttagatggacactacgacgagaagaggaaatccaatgtggaatacacagaggacgagaagaaagccgtgatcgcggctctgaaaaagaaggctttgagcgcctcacagaagtttaggcattccatgaagagggggaggaagagcagcaaggtgatgtccatctcgattctggatgagcgtgaacctgaggaggtgcaggctgtggatgccttccgccagcttcttgtacttgaagagctgctaccatcgcagcatgatgactaccacatgatgctaaggtatgtgatatagtaaaggattgtatgattgcattttcatgtgtggtagcattgctgaaagtttgggatcatgaagatttctcaaggcaagaaagtttgatatcgagaaggcaaagcaaatgtggtctgatatgctgaagtggagaaaggagttcggtgcagataccattctcgaggtaactataatcagatcgagtatttgtaatcatatattactttctaaaacgtcttagataaaatatatatttgtttaactttaaattttggaaaattggataaataaggaaaattttagttatatatctttatttagatccaattgatgtgtacgagatctattggatactctatttttttatttttgcaactttgaatatgacataatttagtcagcttatataaactatctgttttttatgcaagtaatcccagttatatgtatgtgccaaacatactgaaacgtgtacatgcccaacgtggatgcaactctacatacagagaacattacgcggccattttagatcttcaatatatatacgtgacaaccaattatttttattagaaggccctctgaattatctaacacggtattaaatacacacacacacacacattatataaggcgttagtgtgtaacataatttagattaccaaagttcacacaaattgattaacatgttagccattaatattatccgtggatataacttatttcttaattgagtatatattatgtatctaaccattataagacaaaaataccaaaacaaattaaaatatataaaataatttcatccatatataaatagattaaagtattttctcaagggtattcaattgaataccattatttttaccaaaaaagtttatacatacagtatacatatacacaaaaaagagaagcaatcttaggaattatttacaggctattagttcataaacttttgtaaccttttccttttctctaatgcaatcttaggaattcgaattcgaagaagctgataaggtggcagaatgctacaaggttaccatggggttgataaggaaggcaggcctgtctactttgaacggcttggacagatcgatgtgaataggctaatgcaggtcaatggatcgctttgtcaagaaccatgtcaaggagttcgagaagaactttgctgttaagttcccagcttgctcaatcgccgcgaagcaccatattgaccagagcacaacaattcttgacgtgcaaggagtggtaggtatctacaaatttggtggctactcaatggtgcgattttacagtgaataaccaaagacacattttcaggggatgaagcaattcagtaaagctgcaagggagctcattggcatgcttcagaagattgatggtgacaattatccagaggtaatccctttgatatgtgttttgccttcagacattttatctgaattttgtaagcaatattgttcttaccatgccagtttttcttctcttttggtgctagaccctgtgccgcatgttcatcatcaatgcaggccagggattccggcttctatggggcaccgtcaagagctttcttgacccaaagaccactgcaaagattcatgtatttttttcccatcttttatccagttttgctctttagctatgattccaaaactcaattagaatatcgtctccatatttctgtaggttctgggtaacaagtatcagagcaagcttctcgaggtgattgatgctaggtaagaaaataggttacccaattggtagttattagctttactgaactcgtcagctaacttctatggcacatttgtccactgaaatatacacgtttctattattcagtgagttgccagaaatttttggtggaacctgccgatgtgaaggtggttgcatgaaggctgacaaaggcccttggaaggaccccgaaatcatgaaggtgaggactagtccaatatggtcctttgacctgaaccttgccgccttgaatacaaatcaccaaatctttaaggggaaggcactaactcagtattcctaatgcccctttgatgtgaagatggttcaaagtggtgatgggaggtgtggatcactcggtacggcctctttcgaggctccggagaaaatgatttgtgaagacgacacgtatcctaaggtatggaaaaacaaagaaaacaactttcgtgtttgcatagtggccggttgtactcattcctatcattttcttaatgttttttttaaatcaagaaacaagctttgtttgatggggaaacacaattagctggagacgagcattctcagtcacagaaaatttcccgtggccggattgaacatcctcacgtgtcacctcttcacgaggaacttatccccacttcaattcatgtaaggcattcttgttacgattgttgatcactcagataatgaatgaaggcatcaatagtgcaaatattatagttagaatccaaacttacgcggtttgctagctgaaaactcaagcttaatctcaataatgctaacacttgcgacatattcgatctttatttctgggaaacttttttcagacccctggatcaccctattcttgtgatgtcccgatggttgaagaggccatagacgccatctgcaagagccacggaacaccaccagatgagaagattgccatcaccaaaggttagcaccgccactacaagttcatgaatgagcaaacttctgacgaattagtgatactcccagtttcctttcactggtagactgactaaacactatcctttatcagctattataaatgtatcgaatggatccaagcccccactctttgctggcatcatagcacttgtgatgagcatcgcaacgatggtccgtctgacccgcagcatgatgcctgggaaggttctcggtgctgccataggtggagctaccctctcagaaggtaaatcaaaagtacaagagcgccagcggtccaagctatcagaagaggctgtggaggaagctgaagacgccgtctctgcaaagcgcctctcggagcttgaggagaaggtcattgcactcctgacaaaacccgcatcaatgcctgctgataaggaggaggttctgcaggctgctgtctcccgcgttagtgcactggaagaggagcttgcagctacaaagaaggtatcgcctgcaccttgctgggaaatcatgtttttagtaattcgaatcattatgttggtttcgtatattttctgtatccaaaacaataacctgaaacactacgaagtatatgatcctagcacatttctgaacgaattaatctgtttttaaccttgctttgacttgggtctttgcagaccttgcaggagactcttgagcgtcagttggagatcgttgcatacattgagaagaagaagaaaagcaaggtaatgaaatggaggaaaaacatatgacagaacattatgtgccttacacctgtgctcagttcttctggaaaacaaaaacaacttttttcactcaaacataatggtttaattaatactgttatcctagttccacttttttttcccttctggaagcgatgtcatcctagttccacgttcttcttttctggaattgatatgcaaatcaatctggattgacttgatctacgtgctctgaaactacgtttcctgcgctactgcgagttttcactattctcatctcaccaaattaacactgcctttgaactgttcctgcagcgtttctttcgttggtag

SEQ ID NO: 24 - DNA, 4318 bp, Zea mays
  source 1..4318: mol_type = other DNA
  misc_feature 1..4318: gene = Zm00001d016601_B73_P6601_cri-1_T004_V4
atggcagaagtcctatcaggatctcatgaacaccgtctaagctctggtgagtatgcatataattaaatgacatgaccattctcttgctgactgagatggataatatattgcaacagtactttctttctttctttgccctcataaaaaaacttgtgatattcctgtaatgtctgatttttttattgaaacgttgcacttatggcaacacatttttgttttccccaataatcatggacaatttagcataatccatgcaagtcaaattcagtccccgaaattaaacttcacagaattgacttatctagaaatgatatctgcagccttagatggacactacgacgagaagaggaaatccaatgtggaatacacagaggacgagaagaaagccgtgatcgcggctctgaaaaagaaggctttgagcgcctcacagaagtttaggcattccatgaagagggggaggaagagcagcaaggtgatgtccatctcgattctggatgagcgtgaacctgaggaggtgcaggctgtggatgccttccgccagcttcttgtacttgaagagctgctaccatcgcagcatgatgactaccacatgatgctaaggtatgtgatatagtaaaggattgtatgattgcattttcatgtgtggtagcattgctgaaagtttgggatcatgaagatttctcaaggcaagaaagtttgatatcgagaaggcaaagcaaatgtggtctgatatgctgaagtggagaaaggagttcggtgcagataccattctcgaggtaactataatcagatcgagtatttgtaatcatatattactttctaaaacgtcttagataaaatatatatttgtttaactttaaattttggaaaattggataaataaggaaaattttagttatatatctttatttagatccaattgatgtgtacgagatctattggatactctatttttttatttttgcaactttgaatatgacataatttagtcagcttatataaactatctgttttttatgcaagtaatcccagttatatgtatgtgccaaacatactgaaacgtgtacatgcccaacgtggatgcaactctacatacagagaacattacgcggccattttagatcttcaatatatatacgtgacaaccaattatttttattagaaggccctctgaattatctaacacggtattaaatacacacacacacacacattatataaggcgttagtgtgtaacataatttagattaccaaagttcacacaaattgattaacatgttagccattaatattatccgtggatataacttatttcttaattgagtatatattatgtatctaaccattataagacaaaaataccaaaacaaattaaaatatataaaataatttcatccatatataaatagattaaagtattttctcaagggtattcaattgaataccattatttttaccaaaaaagtttatacatacagtatacatatacacaaaaaagagaagcaatcttaggaattatttacaggctattagttcataaacttttgtaaccttttccttttctctaatgcaatcttaggaattcgaattcgaagaagctgataaggtggcagaatgctactcaaggttaccatggggttgataaggaaggcaggcctgtctactttgaacggcttggacagatcgatgtgaataggctaatgcaggtcactacaatggatcgctttgtcaagaaccatgtcaaggagttcgagaagaactttgctgttaagttcccagcttgctcaatcgccgcgaagcaccatattgaccagagcacaacaattcttgacgtgcaaggagtggtaggtatctacaaatttggtggctactcaatggtgcgattttacagtgaataaccaaagacacattttcaggggatgaagcaattcagtaaagctgcaagggagctcattggcatgcttcagaagattgatggtgacaattatccagaggtaatccctttgatatgtgttttgccttcagacattttatctgaattttgtaagcaatattgttcttaccatgccagtttttcttctcttttggtgctagaccctgtgccgcatgttcatcatcaatgcaggccagggattccggcttctatggggcaccgtcaagagctttcttgacccaaagaccactgcaaagattcatgtatttttttcccatcttttatccagttttgctctttagctatgattccaaaactcaattagaatatcgtctccatatttctgtaggttctgggtaacaagtatcagagcaagcttctcgaggtgattgatgctaggtaagaaaataggttacccaattggtagttattagctttactgaactcgtcagctaacttctatggcacatttgtccactgaaatatacacgtttctattattcagtgagttgccagaaatttttggtggaacctgccgatgtgaaggtggttgcatgaaggctgacaaaggcccttggaaggaccccgaaatcatgaaggtgaggactagtccaatatggtcctttgacctgaaccttgccgccttgaatacaaatcaccaaatctttaaggggaaggcactaactcagtattcctaatgcccctttgatgtgaagatggttcaaagtggtgatgggaggtgtggatcactcggtacggcctctttcgaggctccggagaaaatgatttgtgaagacgacacgtatcctaaggtatggaaaaacaaagaaaacaactttcgtgtttgcatagtggccggttgtactcattcctatcattttcttaatgttttttttaaatcaagaaacaagctttgtttgatggggaaacacaattagctggagacgagcattctcagtcacagaaaatttcccgtggccggattgaacatcctcacgtgtcacctcttcacgaggaacttatccccacttcaattcatgtaaggcattcttgttacgattgttgatcactcagataatgaatgaaggcatcaatagtgcaaatattatagttagaatccaaacttacgcggtttgctagctgaaaactcaagcttaatctcaataatgctaacacttgcgacatattcgatctttatttctgggaaacttttttcagacccctggatcaccctattcttgtgatgtcccgatggttgaagaggccatagacgccatctgcaagagccacggaacaccaccagatgagaagattgccatcaccaaaggttagcaccgccactacaagttcatgaatgagcaaacttctgacgaattagtgatactcccagtttcctttcactggtagactgactaaacactatcctttatcagctattataaatgtatcgaatggatccaagcccccactctttgctggcatcatagcacttgtgatgagcatcgcaacgatggtccgtctgacccgcagcatgatgcctgggaaggttctcggtgctgccataggtggagctaccctctcagaaggtaaatcaaaagtacaagagcgccagcggtccaagctatcagaagaggctgtggaggaagctgaagacgccgtctctgcaaagcgcctctcggagcttgaggagaaggtcattgcactcctgacaaaacccgcatcaatgcctgctgataaggaggaggttctgcaggctgctgtctcccgcgttagtgcactggaagaggagcttgcagctacaaagaaggtatcgcctgcaccttgctgggaaatcatgtttttagtaattcgaatcattatgttggtttcgtatattttctgtatccaaaacaataacctgaaacactacgaagtatatgatcctagcacatttctgaacgaattaatctgtttttaaccttgctttgacttgggtctttgcagaccttgcaggagactcttgagcgtcagttggagatcgttgcatacattgagaagaagaagaaaagcaaggtaatgaaatggaggaaaaacatatgacagaacattatgtgccttacacctgtgctcagttcttctggaaaacaaaaacaacttttttcactcaaacataatggtttaattaatactgttatcctagttccacttttttttcccttctggaagcgatgtcatcctagttccacgttcttcttttctggaattgatatgcaaatcaatctggattgacttgatctacgtgctctgaaactacgtttcctgcgctactgcgagttttcactattctcatctcaccaaattaacactgcctttgaactgttcctgcagcgtttctttcgttggtag

SEQ ID NO: 25 - DNA, 4319 bp, Zea mays
  source 1..4319: mol_type = other DNA
  misc_feature 1..4319: gene = Zm00001d016601_B73_P6601_cri-7_T004_V4
atggcagaagtcctatcaggatctcatgaacaccgtctaagctctggtgagtatgcatataattaaatgacatgaccattctcttgctgactgagatggataatatattgcaacagtactttctttctttctttgccctcataaaaaaacttgtgatattcctgtaatgtctgatttttttattgaaacgttgcacttatggcaacacatttttgttttccccaataatcatggacaatttagcataatccatgcaagtcaaattcagtccccgaaattaaacttcacagaattgacttatctagaaatgatatctgcagccttagatggacactacgacgagaagaggaaatccaatgtggaatacacagaggacgagaagaaagccgtgatcgcggctctgaaaaagaaggctttgagcgcctcacagaagtttaggcattccatgaagagggggaggaagagcagcaaggtgatgtccatctcgattctggatgagcgtgaacctgaggaggtgcaggctgtggatgccttccgccagcttcttgtacttgaagagctgctaccatcgcagcatgatgactaccacatgatgctaaggtatgtgatatagtaaaggattgtatgattgcattttcatgtgtggtagcattgctgaaagtttgggatcatgaagatttctcaaggcaagaaagtttgatatcgagaaggcaaagcaaatgtggtctgatatgctgaagtggagaaaggagttcggtgcagataccattctcgaggtaactataatcagatcgagtatttgtaatcatatattactttctaaaacgtcttagataaaatatatatttgtttaactttaaattttggaaaattggataaataaggaaaattttagttatatatctttatttagatccaattgatgtgtacgagatctattggatactctatttttttatttttgcaactttgaatatgacataatttagtcagcttatataaactatctgttttttatgcaagtaatcccagttatatgtatgtgccaaacatactgaaacgtgtacatgcccaacgtggatgcaactctacatacagagaacattacgcggccattttagatcttcaatatatatacgtgacaaccaattatttttattagaaggccctctgaattatctaacacggtattaaatacacacacacacacacattatataaggcgttagtgtgtaacataatttagattaccaaagttcacacaaattgattaacatgttagccattaatattatccgtggatataacttatttcttaattgagtatatattatgtatctaaccattataagacaaaaataccaaaacaaattaaaatatataaaataatttcatccatatataaatagattaaagtattttctcaagggtattcaattgaataccattatttttaccaaaaaagtttatacatacagtatacatatacacaaaaaagagaagcaatcttaggaattatttacaggctattagttcataaacttttgtaaccttttccttttctctaatgcaatcttaggaattcgaattcgaagaagctgataaggtggcagaatgctaccccaaggttaccatggggttgataaggaaggcaggcctgtctactttgaacggcttggacagatcgatgtgaataggctaatgcaggtcactacaatggatcgctttgtcaagaaccatgtcaaggagttcgagaagaactttgctgttaagttcccagcttgctcaatcgccgcgaagcaccatattgaccagagcacaacaattcttgacgtgcaaggagtggtaggtatctacaaatttggtggctactcaatggtgcgattttacagtgaataaccaaagacacattttcaggggatgaagcaattcagtaaagctgcaagggagctcattggcatgcttcagaagattgatggtgacaattatccagaggtaatccctttgatatgtgttttgccttcagacattttatctgaattttgtaagcaatattgttcttaccatgccagtttttcttctcttttggtgctagaccctgtgccgcatgttcatcatcaatgcaggccagggattccggcttctatggggcaccgtcaagagctttcttgacccaaagaccactgcaaagattcatgtatttttttcccatcttttatccagttttgctctttagctatgattccaaaactcaattagaatatcgtctccatatttctgtaggttctgggtaacaagtatcagagcaagcttctcgaggtgattgatgctaggtaagaaaataggttacccaattggtagttattagctttactgaactcgtcagctaacttctatggcacatttgtccactgaaatatacacgtttctattattcagtgagttgccagaaatttttggtggaacctgccgatgtgaaggtggttgcatgaaggctgacaaaggcccttggaaggaccccgaaatcatgaaggtgaggactagtccaatatggtcctttgacctgaaccttgccgccttgaatacaaatcaccaaatctttaaggggaaggcactaactcagtattcctaatgcccctttgatgtgaagatggttcaaagtggtgatgggaggtgtggatcactcggtacggcctctttcgaggctccggagaaaatgatttgtgaagacgacacgtatcctaaggtatggaaaaacaaagaaaacaactttcgtgtttgcatagtggccggttgtactcattcctatcattttcttaatgttttttttaaatcaagaaacaagctttgtttgatggggaaacacaattagctggagacgagcattctcagtcacagaaaatttcccgtggccggattgaacatcctcacgtgtcacctcttcacgaggaacttatccccacttcaattcatgtaaggcattcttgttacgattgttgatcactcagataatgaatgaaggcatcaatagtgcaaatattatagttagaatccaaacttacgcggtttgctagctgaaaactcaagcttaatctcaataatgctaacacttgcgacatattcgatctttatttctgggaaacttttttcagacccctggatcaccctattcttgtgatgtcccgatggttgaagaggccatagacgccatctgcaagagccacggaacaccaccagatgagaagattgccatcaccaaaggttagcaccgccactacaagttcatgaatgagcaaacttctgacgaattagtgatactcccagtttcctttcactggtagactgactaaacactatcctttatcagctattataaatgtatcgaatggatccaagcccccactctttgctggcatcatagcacttgtgatgagcatcgcaacgatggtccgtctgacccgcagcatgatgcctgggaaggttctcggtgctgccataggtggagctaccctctcagaaggtaaatcaaaagtacaagagcgccagcggtccaagctatcagaagaggctgtggaggaagctgaagacgccgtctctgcaaagcgcctctcggagcttgaggagaaggtcattgcactcctgacaaaacccgcatcaatgcctgctgataaggaggaggttctgcaggctgctgtctcccgcgttagtgcactggaagaggagcttgcagctacaaagaaggtatcgcctgcaccttgctgggaaatcatgtttttagtaattcgaatcattatgttggtttcgtatattttctgtatccaaaacaataacctgaaacactacgaagtatatgatcctagcacatttctgaacgaattaatctgtttttaaccttgctttgacttgggtctttgcagaccttgcaggagactcttgagcgtcagttggagatcgttgcatacattgagaagaagaagaaaagcaaggtaatgaaatggaggaaaaacatatgacagaacattatgtgccttacacctgtgctcagttcttctggaaaacaaaaacaacttttttcactcaaacataatggtttaattaatactgttatcctagttccacttttttttcccttctggaagcgatgtcatcctagttccacgttcttcttttctggaattgatatgcaaatcaatctggattgacttgatctacgtgctctgaaactacgtttcctgcgctactgcgagttttcactattctcatctcaccaaattaacactgcctttgaactgttcctgcagcgtttctttcgttggtag

SEQ ID NO: 26 - DNA, 4315 bp, Zea mays
  source 1..4315: mol_type = other DNA
  misc_feature 1..4315: gene = Zm00001d016601_B73_P6601_cri-9_T004_V4
atggcagaagtcctatcaggatctcatgaacaccgtctaagctctggtgagtatgcatataattaaatgacatgaccattctcttgctgactgagatggataatatattgcaacagtactttctttctttctttgccctcataaaaaaacttgtgatattcctgtaatgtctgatttttttattgaaacgttgcacttatggcaacacatttttgttttccccaataatcatggacaatttagcataatccatgcaagtcaaattcagtccccgaaattaaacttcacagaattgacttatctagaaatgatatctgcagccttagatggacactacgacgagaagaggaaatccaatgtggaatacacagaggacgagaagaaagccgtgatcgcggctctgaaaaagaaggctttgagcgcctcacagaagtttaggcattccatgaagagggggaggaagagcagcaaggtgatgtccatctcgattctggatgagcgtgaacctgaggaggtgcaggctgtggatgccttccgccagcttcttgtacttgaagagctgctaccatcgcagcatgatgactaccacatgatgctaaggtatgtgatatagtaaaggattgtatgattgcattttcatgtgtggtagcattgctgaaagtttgggatcatgaagatttctcaaggcaagaaagtttgatatcgagaaggcaaagcaaatgtggtctgatatgctgaagtggagaaaggagttcggtgcagataccattctcgaggtaactataatcagatcgagtatttgtaatcatatattactttctaaaacgtcttagataaaatatatatttgtttaactttaaattttggaaaattggataaataaggaaaattttagttatatatctttatttagatccaattgatgtgtacgagatctattggatactctatttttttatttttgcaactttgaatatgacataatttagtcagcttatataaactatctgttttttatgcaagtaatcccagttatatgtatgtgccaaacatactgaaacgtgtacatgcccaacgtggatgcaactctacatacagagaacattacgcggccattttagatcttcaatatatatacgtgacaaccaattatttttattagaaggccctctgaattatctaacacggtattaaatacacacacacacacacattatataaggcgttagtgtgtaacataatttagattaccaaagttcacacaaattgattaacatgttagccattaatattatccgtggatataacttatttcttaattgagtatatattatgtatctaaccattataagacaaaaataccaaaacaaattaaaatatataaaataatttcatccatatataaatagattaaagtattttctcaagggtattcaattgaataccattatttttaccaaaaaagtttatacatacagtatacatatacacaaaaaagagaagcaatcttaggaattatttacaggctattagttcataaacttttgtaaccttttccttttctctaatgcaatcttaggaattcgaattcgaagaagctgataaggtggcagaatgctaccctcaaggttaccatggggttgataaggaaggcaggcctgtctactttgaacggcttggacagatcgatgtgaataggctaatgcaggtcaatggatcgctttgtcaagaaccatgtcaaggagttcgagaagaactttgctgttaagttcccagcttgctcaatcgccgcgaagcaccatattgaccagagcacaacaattcttgacgtgcaaggagtggtaggtatctacaaatttggtggctactcaatggtgcgattttacagtgaataaccaaagacacattttcaggggatgaagcaattcagtaaagctgcaagggagctcattggcatgcttcagaagattgatggtgacaattatccagaggtaatccctttgatatgtgttttgccttcagacattttatctgaattttgtaagcaatattgttcttaccatgccagtttttcttctcttttggtgctagaccctgtgccgcatgttcatcatcaatgcaggccagggattccggcttctatggggcaccgtcaagagctttcttgacccaaagaccactgcaaagattcatgtatttttttcccatcttttatccagttttgctctttagctatgattccaaaactcaattagaatatcgtctccatatttctgtaggttctgggtaacaagtatcagagcaagcttctcgaggtgattgatgctaggtaagaaaataggttacccaattggtagttattagctttactgaactcgtcagctaacttctatggcacatttgtccactgaaatatacacgtttctattattcagtgagttgccagaaatttttggtggaacctgccgatgtgaaggtggttgcatgaaggctgacaaaggcccttggaaggaccccgaaatcatgaaggtgaggactagtccaatatggtcctttgacctgaaccttgccgccttgaatacaaatcaccaaatctttaaggggaaggcactaactcagtattcctaatgcccctttgatgtgaagatggttcaaagtggtgatgggaggtgtggatcactcggtacggcctctttcgaggctccggagaaaatgatttgtgaagacgacacgtatcctaaggtatggaaaaacaaagaaaacaactttcgtgtttgcatagtggccggttgtactcattcctatcattttcttaatgttttttttaaatcaagaaacaagctttgtttgatggggaaacacaattagctggagacgagcattctcagtcacagaaaatttcccgtggccggattgaacatcctcacgtgtcacctcttcacgaggaacttatccccacttcaattcatgtaaggcattcttgttacgattgttgatcactcagataatgaatgaaggcatcaatagtgcaaatattatagttagaatccaaacttacgcggtttgctagctgaaaactcaagcttaatctcaataatgctaacacttgcgacatattcgatctttatttctgggaaacttttttcagacccctggatcaccctattcttgtgatgtcccgatggttgaagaggccatagacgccatctgcaagagccacggaacaccaccagatgagaagattgccatcaccaaaggttagcaccgccactacaagttcatgaatgagcaaacttctgacgaattagtgatactcccagtttcctttcactggtagactgactaaacactatcctttatcagctattataaatgtatcgaatggatccaagcccccactctttgctggcatcatagcacttgtgatgagcatcgcaacgatggtccgtctgacccgcagcatgatgcctgggaaggttctcggtgctgccataggtggagctaccctctcagaaggtaaatcaaaagtacaagagcgccagcggtccaagctatcagaagaggctgtggaggaagctgaagacgccgtctctgcaaagcgcctctcggagcttgaggagaaggtcattgcactcctgacaaaacccgcatcaatgcctgctgataaggaggaggttctgcaggctgctgtctcccgcgttagtgcactggaagaggagcttgcagctacaaagaaggtatcgcctgcaccttgctgggaaatcatgtttttagtaattcgaatcattatgttggtttcgtatattttctgtatccaaaacaataacctgaaacactacgaagtatatgatcctagcacatttctgaacgaattaatctgtttttaaccttgctttgacttgggtctttgcagaccttgcaggagactcttgagcgtcagttggagatcgttgcatacattgagaagaagaagaaaagcaaggtaatgaaatggaggaaaaacatatgacagaacattatgtgccttacacctgtgctcagttcttctggaaaacaaaaacaacttttttcactcaaacataatggtttaattaatactgttatcctagttccacttttttttcccttctggaagcgatgtcatcctagttccacgttcttcttttctggaattgatatgcaaatcaatctggattgacttgatctacgtgctctgaaactacgtttcctgcgctactgcgagttttcactattctcatctcaccaaattaacactgcctttgaactgttcctgcagcgtttctttcgttggtag

SEQ ID NO: 27 - DNA, 1785 bp, Zea mays
  source 1..1785: mol_type = genomic DNA
  misc_feature 1..1785: gene = NLD
ggggtgtgcggtcgaaggcggcaatggcgagctactcgtcgcggcgtccatgcaatacctgtagcacgaaggcgatggccgggagcgtggtcggcgagcccgtcgtgctggggcagagggtgacggtgctgacggtggacggcggcggcgtccggggtctcatcccgggaaccatcctcgccttcctggaggccaggctgcaggagctggacggaccggaggcgaggctggcggactacttcgactacatcgccggaaccagcaccggcggtctcatcaccgccatgctcaccgcgcccggcaaggacaagcggcctctctacgctgccaaggacatcaactacttttacatggagaactgcccgcgcatcttccctcagaagtgagtccgatgctgccgccattgttctcgcatccatccagcatcgtacgtcctctatacatctgcggatgatcatttgcgcatgtttgtggcatgcatgtgagcaggagcaggcttgcggccgccatgtccgcgctgaggaagccaaagtacaacggcaagtgcatgcgcagcctgattaggagcatcctcggcgagacgagggtaagcgagacgctgaccaacgtcatcatccctgccttcgacatcaggctgctgcagcctatcatcttctctacctacgacgtacgtacgtcgtcacgaatgattcatctgtacgtcgtcgcatgcgaatggctgcctacgccgtgcgctaacatactcagctctttccgatctgctgcgccaatttgcaggccaagagcacgcctctgaagaacgcgctgctctcggacgtgtgcattggcacgtccgccgcgccgacctacctcccggcgcactacttccagactgaagacgccaacggcaaggagcgcgaatacaacctcatcgacggcggtgtggcggccaacaacccggtaactgactagctaactgcaaaacgaacgcacagactccatgtccatggcggcccacaaggtcgatgctaattgttgcttatgtatgtcgcccgattgcacatgcgtagacgatggttgcgatgacgcagatcaccaaaaagatgcttgccagcaaggacaaggccgaggagctgtacccagtgaacccgtcgaactgccgcaggttcctggtgctgtccatcgggacggggtcgacgtccgagcagggcctctacacggcgcggcagtgctcccggtggggcatctgccggtggctccgcaacaacggcatggcccccatcatcgacatcttcatggcggccagctcggacctggtggacatccacgtcgccgcgatgttccagtcgctccacagcgacggcgactacctacgcatccaggacaactcgctccgtggcgccgcggcaaccgtggacgcggcgacgccggagaacatgcggacgctcgtcgggatcggggagcggatgctggcacagcgggtgtccagggtcaacgtggagacagggagcgaggtacgaaccggtgaccggagaaggaagcaatgccgatgccctcggtgggctcgctaggcagctctccgaggagaggagaacaaggctcgcgcgccgcgtctctgccatcaaccccagaagctctagatgtgcgccctacgatatctaagacaagtggctttactgtcaatcacatgcttgtaaataagtagactttattttaataaaatataaatatatatatattctgataaccaagattcgaaccctcacttatacacaattttatcttattttttataaaacgtgaacg